European Patent Application EP 4 599 840 A1, published August 13, 2025. Title: Antimicrobial proteins. Applicant: The Olive Feed Corporation Limited. Application EP. The sequence listing filed with the application follows.

SEQUENCE LISTING (12 sequences)

SEQ ID NO: 1 - protein, 47 aa, Olea europaea
RTCESQSHRFKGSCVSKSNCAAVCQTEGFPDGYCRGFRRRCFCSKHC

SEQ ID NO: 2 - protein, 50 aa, Olea europaea
RVCSRLSKTWSGLCLNSGNCNRQCRNWEGALRGACHKRGWGFACFCYRKC

SEQ ID NO: 3 - DNA, 145 bp, Olea europaea
  source 1..145: mol_type = genomic DNA
aggacttgtgaatcccaaagccaccggttcaagggatcttgtgttagtaaaagcaactgcgcggcggtttgccagactgagggatttcccgacggctattgcaggggctttcgccgccgctgcttctgctccaaacattgttaaa

SEQ ID NO: 4 - DNA, 148 bp, synthetic construct
  source 1..148: mol_type = other DNA
tgacggacatgcgagtcacagagtcatagatttaaaggtagttgcgtcagcaagtcaaattgtgccgctgtgtgtcaaacagaaggtttccctgatgggtactgtcgcgggttccgtagacgttgtttctgttctaagcactgctgaa

SEQ ID NO: 5 - DNA, 150 bp, Olea europaea
  source 1..150: mol_type = genomic DNA
agagtttgttcgaggctgagcaagacatggtctggattatgcctgaactccgggaactgcaaccggcagtgcaggaactgggagggggctctgcgtggagcttgtcacaaaaggggctggggattcgcttgcttttgctaccggaaatgc

SEQ ID NO: 6 - DNA, 150 bp, synthetic construct
  source 1..150: mol_type = other DNA
cgtgtctgttcgcgactctccaaaacgtggtccggtctttgtctgaattctggcaactgcaatcgccagtgtagaaactgggaaggtgcattaagaggtgcttgtcataagcgtggttggggtttcgcgtgcttttgctatcgtaaatgc

SEQ ID NO: 7 - DNA, 32 bp, synthetic construct
  source 1..32: mol_type = other DNA
attctagagctaatacgtgcaacaaaccccga

SEQ ID NO: 8 - DNA, 22 bp, synthetic construct
  source 1..22: mol_type = other DNA
aggattgggtaatttgcgcgcc

SEQ ID NO: 9 - DNA, 28 bp, synthetic construct
  source 1..28: mol_type = other DNA
tatgcagctgtgttcttcatgctcatgc

SEQ ID NO: 10 - DNA, 25 bp, synthetic construct
  source 1..25: mol_type = other DNA
acaatgtttggagcagaagcagcgg

SEQ ID NO: 11 - DNA, 33 bp, synthetic construct
  source 1..33: mol_type = other DNA
tatcctagcttatttgcaactgctatgctcgtg

SEQ ID NO: 12 - DNA, 24 bp, synthetic construct
  source 1..24: mol_type = other DNA
acagtgtttggtgcagaaacagcg